European Patent Specification EP 3 535 294 B1, published February 12, 2025. Title: ANTI-FAMILY WITH SEQUENCE SIMILARITY 19, MEMBER A5 ANTIBODIES AND METHOD OF USE THEREOF. Applicant: NEURACLE SCIENCE CO., LTD. The sequence listing filed with the application follows.

SEQUENCE LISTING (166 sequences)

SEQ ID NO: 1 - protein, 132 aa, Homo Sapiens
MAPSPRTGSRQDATALPSMSSTFWAFMILASLLIAYCSQLAAGTCEIVTLDRDSSQPRRTIARQTARCACRKGQIAGTTRARPACVDARIIKTKQWCDMLPCLEGEGCDLLINRSGWTCTQPGGRIKTTTVS

SEQ ID NO: 2 - protein, 20 aa, Artificial Sequence
  Epitope F5
CDMLPCLEGEGCDLLINRSG

SEQ ID NO: 3 - DNA, 1501 bp, Homo Sapiens
ggcggcggaggatggcgcgcgcggggcccgcacgtggaggccggcgcgggggcgcgggcagggccggctgctgagacgcgctgctgccccccgcgcgggcgccgcggcttcaatggcgccatcgcccaggaccggcagccggcaagatgcgaccgccctgcccagcatgtcctcaactttctgggcgttcatgatcctggccagcctgctcatcgcctactgcagtcagctggccgccggcacctgtgagattgtgaccttggaccgggacagcagccagcctcggaggacgatcgcccggcagaccgcccgctgtgcgtgtagaaaggggcagatcgccggcaccacgagagcccggcccgcctgtgtggacgcaagaatcatcaagaccaagcagtggtgtgacatgcttccgtgtctggagggggaaggctgcgacttgttaatcaaccggtcaggctggacgtgcacgcagcccggcgggaggataaagaccaccacggtctcctgacaaacacagcccctgagggggccccgggagtggccttggctccctggagagcccacgtctcagccacagttctccactcgcctcggacttcacccgttctctgccgcccgcccactccgtttccctgtggtccgtgaaggacggcctcaggccttggcatcctgagcttcggtctgtccagccgacccgaggaggccggactcagacacataggcggggggcggcacctggcatcagcaatacgcagtctgtgggagcccggccgcgcccagcccccgccgaccgtggcgttggccctgctgtcctcagaggaggaggaggaggaggcagctccggcagccacagaaggctgcagcccagcccgcctgagacacgacgcctgccccaggggactgtcaggcacagaagcggcctcctcccgtgccccagactgtccgaattgcttttattttcttatactttcagtatactccatagaccaaagagcaaaatctatctgaacctggacgcaccctcactgtcagggtccctggggtcgcttgtgcgggcgggagggcaatggtggcagagacatgctggtggccccggcggagcggagagggcggccgtggtggaggcctccaccccaggagcaccccgcacaccctcggaggacgggcttcggctgcgcggaggccgtggcacacctgcgggaggcagcgacggcccccacgcagacgccgggaacgcaggccgctttattcctctgtacttagatcaacttgaccgtactaaaatccctttctgttttaaccagttaaacatgcctcttctacagctccatttttgatagttggataatccagtatctgccaagagcatgttgggtctcccgtgactgctgcctcatcgataccccatttagctccagaaagcaaagaaaactcgagtaacacttgtttgaaagagatcattaaatgtattttgcaaagcccaaaaaaaaaaaaaaaa

SEQ ID NO: 4 - protein, 125 aa, Homo Sapiens
MQLLKALWALAGAALCCFLVLVIHAQFLKEGQLAAGTCEIVTLDRDSSQPRRTIARQTARCACRKGQIAGTTRARPACVDARIIKTKQWCDMLPCLEGEGCDLLINRSGWTCTQPGGRIKTTTVS

SEQ ID NO: 5 - protein, 122 aa, Artificial Sequence
  1-65 Antibody VH
AVTLDESGGGLQTPGGALSLVCKASGFTFSSYQMGWVRQAPGKGLEWVGVINKSGSDTSYGSAVKGRATISRDNGQSTVRLQLNNLRAEDTGTYFCAKGSASYITAATIDAWGHGTEVIVSS

SEQ ID NO: 6 - protein, 110 aa, Artificial Sequence
  1-65 Antibody VL
ALTQPSSVSANPGETVKITCSGGGSSGYGYGWYQQKSPSSAPLTVIYWNDKRPSDIPSRFSGSKSGSTHTLTITGVQAEDEAVYFCGNDDYSSDSGYVGVFGAGTTLTVL

SEQ ID NO: 7 - protein, 5 aa, Artificial Sequence
  1-65 Antibody VH-CDR1
SYQMG

SEQ ID NO: 8 - protein, 10 aa, Artificial Sequence
  1-65 Antibody VH-CDR2
VINKSGSDTS

SEQ ID NO: 9 - protein, 13 aa, Artificial Sequence
  1-65 Antibody VH-CDR3
GSASYITAATIDA

SEQ ID NO: 10 - protein, 11 aa, Artificial Sequence
  1-65 Antibody VL-CDR1
SGGGSSGYGYG

SEQ ID NO: 11 - protein, 7 aa, Artificial Sequence
  1-65 Antibody VL-CDR2
WNDKRPS

SEQ ID NO: 12 - protein, 14 aa, Artificial Sequence
  1-65 Antibody VL-CDR3
GNDDYSSDSGYVGV

SEQ ID NO: 13 - protein, 14 aa, Artificial Sequence
  Epitope F1
QLAAGTCEIVTLDR

SEQ ID NO: 14 - protein, 20 aa, Artificial Sequence
  Epitope F2
TLDRDSSQPRRTIARQTARC

SEQ ID NO: 15 - protein, 20 aa, Artificial Sequence
  Epitope F3
TARCACRKGQIAGTTRARPA

SEQ ID NO: 16 - protein, 20 aa, Artificial Sequence
  Epitope F4
ARPACVDARIIKTKQWCDML

SEQ ID NO: 17 - protein, 20 aa, Artificial Sequence
  Epitope F6
NRSGWTCTQPGGRIKTTTVS

SEQ ID NO: 18 - DNA, 366 bp, Artificial Sequence
  1-65 Antibody VH
gccgtgacactggacgaatctgggggagggctgcagactccaggcggagctctgagcctggtgtgcaaggcatccgggttcacctttagctcctaccagatgggatgggtgcggcaggcaccagggaagggcctggagtgggtcggagtgatcaacaaatctgggagtgacacaagctacggcagcgccgtgaagggaagggccaccatcagcagggacaatggccagagtaccgtgcggctgcagctgaacaatctgcgcgctgaggacactggcacctacttctgtgctaagggatcagcaagctatatcacagccgctactattgatgcatggggacacgggacagaagtcatcgtgtctagt

SEQ ID NO: 19 - DNA, 330 bp, Artificial Sequence
  1-65 Antibody VL
gccctgactcagccctcttccgtgtcagccaaccctggagaaactgtgaagatcacctgcagcggaggagggagctccggatacggatatgggtggtatcagcagaaatccccatctagtgcccccctgactgtgatctattggaacgacaagaggcctagtgatattccatcaagattcagtggatcaaaaagcgggtccactcacaccctgacaatcactggcgtgcaggcagaggacgaagccgtctacttctgcggaaatgacgattactcaagcgattctggctatgtgggcgtctttggcgcaggaaccacactgacagtgctg

SEQ ID NO: 20-25 - skipped (6 entries)

SEQ ID NO: 26 - protein, 53 aa, Homo Sapiens
MYHHREWPARIIKTKQWCDMLPCLEGEGCDLLINRSGWTCTQPGGRIKTTTVS

SEQ ID NO: 27 - protein, 452 aa, Artificial Sequence
  1-65 Antibody HC
AVTLDESGGGLQTPGGALSLVCKASGFTFSSYQMGWVRQAPGKGLEWVGVINKSGSDTSYGSAVKGRATISRDNGQSTVRLQLNNLRAEDTGTYFCAKGSASYITAATIDAWGHGTEVIVSSASTKGPSVFPLAPSSKSTSGGTAALGCLVKDYFPEPVTVSWNSGALTSGVHTFPAVLQSSGLYSLSSVVTVPSSSLGTQTYICNVNHKPSNTKVDKKVEPKSCDKTHTCPPCPAPELLGGPSVFLFPPKPKDTLMISRTPEVTCVVVDVSHEDPEVKFNWYVDGVEVHNAKTKPREEQYNSTYRVVSVLTVLHQDWLNGKEYKCKVSNKALPAPIEKTISKAKGQPREPQVYTLPPSREEMTKNQVSLTCLVKGFYPSDIAVEWESNGQPENNYKTTPPVLDSDGSFFLYSKLTVDKSRWQQGNVFSCSVMHEALHNHYTQKSLSLSPGK

SEQ ID NO: 28 - protein, 217 aa, Artificial Sequence
  1-65 Antibody LC
ALTQPSSVSANPGETVKITCSGGGSSGYGYGWYQQKSPSSAPLTVIYWNDKRPSDIPSRFSGSKSGSTHTLTITGVQAEDEAVYFCGNDDYSSDSGYVGVFGAGTTLTVLRSVAAPSVFIFPPSDEQLKSGTASVVCLLNNFYPREAKVQWKVDNALQSGNSQESVTEQDSKDSTYSLSSTLTLSKADYEKHKVYACEVTHQGLSSPVTKSFNRGEC

SEQ ID NO: 29 - protein, 5 aa, Artificial Sequence
  P2-C12  antibody VH CDR1
TYAVT

SEQ ID NO: 30 - protein, 16 aa, Artificial Sequence
  P2-C12 antibody VH CDR2
YINWRGGTSYANWAKG

SEQ ID NO: 31 - protein, 15 aa, Artificial Sequence
  P2-C12 antibody VH CDR3
DASSGAAFGSYGMDP

SEQ ID NO: 32 - protein, 11 aa, Artificial Sequence
  P2-C12  antibody VL CDR1
QASQSISSYLS

SEQ ID NO: 33 - protein, 7 aa, Artificial Sequence
  P2-C12 antibody VL CDR2
EASKLAS

SEQ ID NO: 34 - protein, 12 aa, Artificial Sequence
  P2-C12 antibody VL CDR3
QQGYSSTNVWNA

SEQ ID NO: 35 - protein, 6 aa, Artificial Sequence
  13B4 antibody VH CDR1
SSNWWS

SEQ ID NO: 36 - protein, 16 aa, Artificial Sequence
  13B4 antibody VH CDR2
EIYHGGTTNYNPSLKG

SEQ ID NO: 37 - protein, 9 aa, Artificial Sequence
  13B4 antibody VH CDR3
WQLVGGLDV

SEQ ID NO: 38 - protein, 11 aa, Artificial Sequence
  13B4 antibody VL CDR1
SGDKLGNVYAS

SEQ ID NO: 39 - protein, 7 aa, Artificial Sequence
  13B4 antibody VL CDR2
QDNKRPS

SEQ ID NO: 40 - protein, 9 aa, Artificial Sequence
  13B4 antibody VL CDR3
QAWDSSTAV

SEQ ID NO: 41 - protein, 5 aa, Artificial Sequence
  13F7 antibody VH CDR1
GYSWT

SEQ ID NO: 42 - protein, 16 aa, Artificial Sequence
  13F7 antibody VH CDR2
EISHFGSANYNPSLKS

SEQ ID NO: 43 - protein, 15 aa, Artificial Sequence
  13F7 antibody VH CDR3
ALRGTYSRFYYGMDV

SEQ ID NO: 44 - protein, 16 aa, Artificial Sequence
  13F7 antibody VL CDR1
RSSQSLLHSNGYNYLD

SEQ ID NO: 45 - protein, 7 aa, Artificial Sequence
  13F7 antibody VL CDR2
LGSNRAS

SEQ ID NO: 46 - protein, 9 aa, Artificial Sequence
  13F7 antibody VL CDR3
MQARQTPLT

SEQ ID NO: 47 - protein, 5 aa, Artificial Sequence
  15A9 antibody VH CDR1
SYYWS

SEQ ID NO: 48 - protein, 16 aa, Artificial Sequence
  15A9 antibody VH CDR2
YIYPSGSTNYNPSLKS

SEQ ID NO: 49 - protein, 12 aa, Artificial Sequence
  15A9 antibody VH CDR3
VNPFGYYYAMDV

SEQ ID NO: 50 - protein, 11 aa, Artificial Sequence
  15A9 antibody VL CDR1
RASQSISTSLN

SEQ ID NO: 51 - protein, 7 aa, Artificial Sequence
  15A9 antibody VL CDR2
GASTLQS

SEQ ID NO: 52 - protein, 9 aa, Artificial Sequence
  15A9 antibody VL CDR3
QESASIPRT

SEQ ID NO: 53 - protein, 5 aa, Artificial Sequence
  P1-A03 antibody VH CDR1
SDYMS

SEQ ID NO: 54 - protein, 16 aa, Artificial Sequence
  P1-A03 antibody VH CDR2
IIYPSTTTYYASWAKG

SEQ ID NO: 55 - protein, 10 aa, Artificial Sequence
  P1-A03 antibody VH CDR3
GSNWSSGMNL

SEQ ID NO: 56 - protein, 11 aa, Artificial Sequence
  P1-A03 antibody VL CDR1
LASEDIYSGIS

SEQ ID NO: 57 - protein, 7 aa, Artificial Sequence
  P1-A03 antibody VL CDR2
GASNLES

SEQ ID NO: 58 - protein, 12 aa, Artificial Sequence
  P1-A03 antibody VL CDR3
LGGYSYSSTGLT

SEQ ID NO: 59 - protein, 5 aa, Artificial Sequence
  P1-A08 antibody VH CDR1
TYYMS

SEQ ID NO: 60 - protein, 16 aa, Artificial Sequence
  P1-A08 antibody VH CDR2
IVYPSGTTYYANWAKG

SEQ ID NO: 61 - protein, 8 aa, Artificial Sequence
  P1-A08 antibody VH CDR3
GDSFGYGL

SEQ ID NO: 62 - protein, 11 aa, Artificial Sequence
  P1-A08 antibody VL CDR1
TADTLSRSYAS

SEQ ID NO: 63 - protein, 7 aa, Artificial Sequence
  P1-A08 antibody VL CDR2
RDTSRPS

SEQ ID NO: 64 - protein, 13 aa, Artificial Sequence
  P1-A08 antibody VL CDR3
ATSDGSGSNYQYV

SEQ ID NO: 65 - protein, 5 aa, Artificial Sequence
  P1-F02 antibody VH CDR1
NYYMG

SEQ ID NO: 66 - protein, 16 aa, Artificial Sequence
  P1-F02 antibody VH CDR2
IIYASGSTYYASWAKG

SEQ ID NO: 67 - protein, 17 aa, Artificial Sequence
  P1-F02 antibody VH CDR3
IDIGVGDYGWAYDRLDL

SEQ ID NO: 68 - protein, 11 aa, Artificial Sequence
  P1-F02 antibody VL CDR1
LASEDIYSGIS

SEQ ID NO: 69 - protein, 7 aa, Artificial Sequence
  P1-F02 antibody VL CDR2
GASNLES

SEQ ID NO: 70 - protein, 10 aa, Artificial Sequence
  P1-F02 antibody VL CDR3
LGGYSYSSIT

SEQ ID NO: 71 - protein, 5 aa, Artificial Sequence
  P2-A01 antibody VH CDR1
GYYMS

SEQ ID NO: 72 - protein, 16 aa, Artificial Sequence
  P2-A01 antibody VH CDR2
IIYPSGSTDYASWAKG

SEQ ID NO: 73 - protein, 15 aa, Artificial Sequence
  P2-A01 antibody VH CDR3
VAGYVGYGYETFFDI

SEQ ID NO: 74 - protein, 11 aa, Artificial Sequence
  P2-A01 antibody VL CDR1
LASEDIYSGIS

SEQ ID NO: 75 - protein, 7 aa, Artificial Sequence
  P2-A01 antibody VL CDR2
GASNLES

SEQ ID NO: 76 - protein, 14 aa, Artificial Sequence
  P2-A01 antibody VL CDR3
LGGVTYSSTGTHLT

SEQ ID NO: 77 - protein, 5 aa, Artificial Sequence
  P2-A03 antibody VH CDR1
NYDMS

SEQ ID NO: 78 - protein, 16 aa, Artificial Sequence
  P2-A03 antibody VH CDR2
FMDTDGSAYYATWAKG

SEQ ID NO: 79 - protein, 11 aa, Artificial Sequence
  P2-A03 antibody VH CDR3
RGSSYYGGIDI

SEQ ID NO: 80 - protein, 11 aa, Artificial Sequence
  P2-A03 antibody VL CDR1
QASQSIGGNLA

SEQ ID NO: 81 - protein, 7 aa, Artificial Sequence
  P2-A03 antibody VL CDR2
RASTLAS

SEQ ID NO: 82 - protein, 14 aa, Artificial Sequence
  P2-A03 antibody VL CDR3
QSPAYDPAAYVGNA

SEQ ID NO: 83 - protein, 5 aa, Artificial Sequence
  P2-F07 antibody VH CDR1
SYYMN

SEQ ID NO: 84 - protein, 16 aa, Artificial Sequence
  P2-F07 antibody VH CDR2
IIYPSGTTYYAGWAKG

SEQ ID NO: 85 - protein, 8 aa, Artificial Sequence
  P2-F07 antibody VH CDR3
TVSGYFDI

SEQ ID NO: 86 - protein, 11 aa, Artificial Sequence
  P2-F07 antibody VL CDR1
LASEDIYSALA

SEQ ID NO: 87 - protein, 7 aa, Artificial Sequence
  P2-F07 antibody VL CDR2
GTSNLES

SEQ ID NO: 88 - protein, 9 aa, Artificial Sequence
  P2-F07 antibody VL CDR3
QGYSSYPLT

SEQ ID NO: 89 - protein, 5 aa, Artificial Sequence
  P2-F11 antibody VH CDR1
SYGVS

SEQ ID NO: 90 - protein, 16 aa, Artificial Sequence
  P2-F11 antibody VH CDR2
YIANNYNPHYASWAKG

SEQ ID NO: 91 - protein, 7 aa, Artificial Sequence
  P2-F11 antibody VH CDR3
DNYGMDP

SEQ ID NO: 92 - protein, 13 aa, Artificial Sequence
  P2-F11 antibody VL CDR1
QASQSVYNNKNLA

SEQ ID NO: 93 - protein, 7 aa, Artificial Sequence
  P2-F11 antibody VL CDR2
AASTLAS

SEQ ID NO: 94 - protein, 13 aa, Artificial Sequence
  P2-F11 antibody VL CDR3
QGEFSCSSADCNA

SEQ ID NO: 95 - protein, 100 aa, Artificial Sequence
  M1 mutant
QFLKEGQLAAGTCEVIAAHRDSSQPRRTIARQTARCACRKGQIAGTTRARPACVDARIIKTKQWCDMLPCLEGEGCDLLINRSGWTCTQPGGRIKTTTVS

SEQ ID NO: 96 - protein, 100 aa, Artificial Sequence
  M2 mutant
QFLKEGQLAAGTCEIVTLDRCCNKNRRTIARQTARCACRKGQIAGTTRARPACVDARIIKTKQWCDMLPCLEGEGCDLLINRSGWTCTQPGGRIKTTTVS

SEQ ID NO: 97 - protein, 100 aa, Artificial Sequence
  M3 mutant
QFLKEGQLAAGTCEIVTLDRDSSQPRIEERSQTARCACRKGQIAGTTRARPACVDARIIKTKQWCDMLPCLEGEGCDLLINRSGWTCTQPGGRIKTTTVS

SEQ ID NO: 98 - protein, 100 aa, Artificial Sequence
  M4 mutant
QFLKEGQLAAGTCEIVTLDRDSSQPRRTIARQTVKCSCFPGQIAGTTRARPACVDARIIKTKQWCDMLPCLEGEGCDLLINRSGWTCTQPGGRIKTTTVS

SEQ ID NO: 99 - protein, 100 aa, Artificial Sequence
  M5 mutant
QFLKEGQLAAGTCEIVTLDRDSSQPRRTIARQTARCACRKGQIAGTTRNKPSCVDARIIKTKQWCDMLPCLEGEGCDLLINRSGWTCTQPGGRIKTTTVS

SEQ ID NO: 100 - protein, 100 aa, Artificial Sequence
  M6 mutant
QFLKEGQLAAGTCEIVTLDRDSSQPRRTIARQTARCACRKGQIAGTTRARPACVDARIILQRWWCQMELCLEGEGCDLLINRSGWTCTQPGGRIKTTTVS

SEQ ID NO: 101 - protein, 100 aa, Artificial Sequence
  M7 mutant
QFLKEGQLAAGTCEIVTLDRDSSQPRRTIARQTARCACRKGQIAGTTRARPACVDARIIKTKQWCDMLPCLEGEECKTLPDNSGWTCTQPGGRIKTTTVS

SEQ ID NO: 102 - protein, 101 aa, Artificial Sequence
  M8 mutant
QFLKEGQLAAGTCEIVTLDRDSSQPRRTIARQTARCACRKGQIAGTTRARPACVDARIIKTKQWCDMLPCLEGEGCDLLINRSGWTCSCSSGNKIKTTTVS

SEQ ID NO: 103 - protein, 121 aa, Artificial Sequence
  P2-C12 antibody VH
QSLEESGGRLVTPGTPLTLTCTVSGFSLSTYAVTWVRQAPGKGLEWIGYINWRGGTSYANWAKGRFTISKTSSTTVDLKMTSPTTEDTATYFCARDASSGAAFGSYGMDPWGPGTLVTVSS

SEQ ID NO: 104 - protein, 118 aa, Artificial Sequence
  13B4 antibody VH
QVQLQESGPGLVKPSGTLSLNCAVSGGSISSSNWWSWVRQPPGKGLEWIGEIYHGGTTNYNPSLKGRVTMSVDKTKNQFSLRLSSVTAVDTAVYYCARWQLVGGLDVWGQGTTVTVSS

SEQ ID NO: 105 - protein, 123 aa, Artificial Sequence
  13F7 antibody VH
QVQLQEWGAGLLKPSETLSLTCAINAESFNGYSWTWIRQTPGKGLEWIGEISHFGSANYNPSLKSRATISADKSKNQFSLKLTSVTAVDTAVYYCARALRGTYSRFYYGMDVWGQGTTVTVSS

SEQ ID NO: 106 - protein, 120 aa, Artificial Sequence
  15A9 antibody VH
QVQLQESGPGLVKPSETLSLTCTVSGGSISSYYWSWIRQPPGKGLEWIGYIYPSGSTNYNPSLKSRVTISVDTSKNQFSLNLKSVTAVDTAVYYCARVNPFGYYYAMDVWGQGTTVTVSS

SEQ ID NO: 107 - protein, 116 aa, Artificial Sequence
  P1-A03 antibody VH
QSVEESGGRLVTPGTPLTLTCTVSGFSLSSDYMSWVRQAPGEGLEWIGIIYPSTTTYYASWAKGRFTISKTSSTTVELKMTSLTTEDTATYFCARGSNWSSGMNLWGPGTLVTVSS

SEQ ID NO: 108 - protein, 113 aa, Artificial Sequence
  P1-A08 antibody VH
QSLEESGGRLVTPGTPLTLTCTASGFSLSTYYMSWVRQAPGKGLEWIGIVYPSGTTYYANWAKGRFTISTASTTVDLMITSPTTEDTATYFCARGDSFGYGLWGPGTLVTVSS

SEQ ID NO: 109 - protein, 122 aa, Artificial Sequence
  P1-F02 antibody VH
QSLEESGGRLVTPGTPLTLTCTASGFSLSNYYMGWVRQAPGEGLEWIGIIYASGSTYYASWAKGRFTISKTSTTVDLKMTSLTTEDTATYFCARIDIGVGDYGWAYDRLDLWGQGTLVTVSS

SEQ ID NO: 110 - protein, 121 aa, Artificial Sequence
  P2-A01 antibody VH
QEQLVESGGRLVTPGTPLTLSCTASGFFLSGYYMSWVRQAPGKGLEWIGIIYPSGSTDYASWAKGRFTISKTSTTVDLKITTPTTEDTATYFCARVAGYVGYGYETFFDIWGPGTLVTVSL

SEQ ID NO: 111 - protein, 116 aa, Artificial Sequence
  P2-A03 antibody VH
QSVEESGGRLVTPGTPLTLTCTVSGFSLNNYDMSWVRQAPGKGLEYIGFMDTDGSAYYATWAKGRFTISRTSTTVDLKMTSPTTEDTATYFCARRGSSYYGGIDIWGPGTPVTVSL

SEQ ID NO: 112 - protein, 113 aa, Artificial Sequence
  P2-F07 antibody VH
QSLEESGGRLVTPGTPLTLTCTASGFSLSSYYMNWVRQAPGKGLEWIGIIYPSGTTYYAGWAKGRFTISKTSTTVDLKITSPTSEDTATYFCARTVSGYFDIWGPGTLVTVSL

SEQ ID NO: 113 - protein, 114 aa, Artificial Sequence
  P2-F11 antibody VH
QEQLVESGGRLVTPGTTLTLTCTVSGFSLSSYGVSWVRQAPGKGLEWIGYIANNYNPHYASWAKGRFTISKTSSTTVDLKMTSLTTEDTATYFCARDNYGMDPWGPGTLVTVSS

SEQ ID NO: 114 - protein, 110 aa, Artificial Sequence
  P2-C12 antibody VL
ELDMTQTPSSVSAAVGGTVTIKCQASQSISSYLSWYQQKPGQPPKLLIYEASKLASGVPSRFSGSGYGTEFTLTISDLECADAATYYCQQGYSSTNVWNAFGGGTNVEIK

SEQ ID NO: 115 - protein, 106 aa, Artificial Sequence
  13B4 antibody VL
SYELTQPLSVSVSPGQTASITCSGDKLGNVYASWYQQKPGQSPTLVIYQDNKRPSGIPERFSGSNSGKTATLTISGTQALDEADYYCQAWDSSTAVFGGGTKLTVL

SEQ ID NO: 116 - protein, 112 aa, Artificial Sequence
  13F7 antibody VL
DIVMTQTPLSLPVAPGEPASISCRSSQSLLHSNGYNYLDWYVQKPGQPPQLLIYLGSNRASGVPDRFSGSGSGTDFTLKISRVEAEDVGVYYCMQARQTPLTFGGGTKVEIK

SEQ ID NO: 117 - protein, 107 aa, Artificial Sequence
  15A9 antibody VL
DIQMTQSPSSLSASVGDRITISCRASQSISTSLNWYQQTPGKAPRLLIYGASTLQSGVPSRFSGGGSGTDFSLTITSLQPEDFATYYCQESASIPRTFGQGTKLDIK

SEQ ID NO: 118 - protein, 110 aa, Artificial Sequence
  P1-A03 antibody VL
ELVMTQTPPSLSASVGETVRIRCLASEDIYSGISWYQQKPEKPPTLLISGASNLESGVPPRFSGSGSGTDYTLTIGGVQAEDAATYYCLGGYSYSSTGLTFGAGTNVEIK

SEQ ID NO: 119 - protein, 110 aa, Artificial Sequence
  P1-A08 antibody VL
ELVLTQSPSVQVNLGQTVSLTCTADTLSRSYASWYQQKPGQAPVLLIYRDTSRPSGVPDRFSGSSSGNTATLTISGAQAGDEADYYCATSDGSGSNYQYVFGGGTQLTVT

SEQ ID NO: 120 - protein, 108 aa, Artificial Sequence
  P1-F02 antibody VL
ELDMTQTPPSLSASVGETVRIRCLASEDIYSGISWYQQKPGKPPTLLIYGASNLESGVPPRFSGSGSGTDYTLTIGGVQAEDAATYYCLGGYSYSSITFGAGTNVEIK

SEQ ID NO: 121 - protein, 112 aa, Artificial Sequence
  P2-A01 antibody VL
ELVMTQTPPSLSASVGETVRIRCLASEDIYSGISWYQQKPGKPPTLLIYGASNLESGVPPRFSGSGSGSDYTLTIGGVQAEDAATYYCLGGVTYSSTGTHLTFGAGTNVEIK

SEQ ID NO: 122 - protein, 112 aa, Artificial Sequence
  P2-A03 antibody VL
ELDLTQTPASVSEPVGGTVTIKCQASQSIGGNLAWYQQKPGQPPKLLIYRASTLASGVPSRFKGSGSGTDFTLTISDLECADAATYYCQSPAYDPAAYVGNAFGGGTELEIL

SEQ ID NO: 123 - protein, 107 aa, Artificial Sequence
  P2-F07 antibody VL
ELDLTQTPPSLSASVGGTVTINCLASEDIYSALAWYQQKPGKPPTLLISGTSNLESGVPPRFSGSGSGTDYTLTIGGVQAEDAATYFCQGYSSYPLTFGAGTNVEIK

SEQ ID NO: 124 - protein, 113 aa, Artificial Sequence
  P2-F11 antibody VL
ELDLTQTPSSVSAAVGGTVTINCQASQSVYNNKNLAWYQQKPGQPPKLLIYAASTLASGVSSRFKGSGSGTQFTLTISDVQCDDAATYYCQGEFSCSSADCNAFGGGTELEIL

SEQ ID NO: 125 - protein, 20 aa, Artificial Sequence
  F5
SDMLPSLEGEGSDLLINRSG

SEQ ID NO: 126 - protein, 20 aa, Artificial Sequence
  F5-1 (#1)
SDMLPSLEGEASDLLINRSG

SEQ ID NO: 127 - protein, 20 aa, Artificial Sequence
  F5-2 (#2)
SDMLPSLEGEGSALLINRSG

SEQ ID NO: 128 - protein, 20 aa, Artificial Sequence
  F5-3 (#3)
SDMLPSLEGEGSDALINRSG

SEQ ID NO: 129 - protein, 20 aa, Artificial Sequence
  F5-4 (#4)
SDMLPSLEGEGSDLLANRSG

SEQ ID NO: 130 - protein, 20 aa, Artificial Sequence
  F5-5 (#5)
SDMLPSLAGEGSDLLINRSG

SEQ ID NO: 131 - protein, 20 aa, Artificial Sequence
  F5-6 (#6)
SDMLPSLEGAGSDLLINRSG

SEQ ID NO: 132 - protein, 20 aa, Artificial Sequence
  F5-7 (#7)
SDMLPSLEGEGSDLLIARSG

SEQ ID NO: 133 - protein, 20 aa, Artificial Sequence
  F5-8 (#8)
SDMLPSLEGEGSDLLINASG

SEQ ID NO: 134 - protein, 5 aa, Artificial Sequence
  EP1 Epitope
IVTLD

SEQ ID NO: 135 - protein, 5 aa, Artificial Sequence
  EP2 Epitope
DSSQP

SEQ ID NO: 136 - protein, 5 aa, Artificial Sequence
  EP3 Epitope
RTIAR

SEQ ID NO: 137 - protein, 7 aa, Artificial Sequence
  EP4 Epitope
ARCACRK

SEQ ID NO: 138 - protein, 4 aa, Artificial Sequence
  EP5 Epitope
ARPA

SEQ ID NO: 139 - protein, 9 aa, Artificial Sequence
  EP6 Epitope
KTKQWCDML

SEQ ID NO: 140 - protein, 8 aa, Artificial Sequence
  EP7 Epitope
GCDLLINR

SEQ ID NO: 141 - protein, 8 aa, Artificial Sequence
  EP8 Epitope
TCTQPGGR

SEQ ID NO: 142 - protein, 100 aa, Artificial Sequence
  Wild-type FAM19A5 Isoform 2 (no signal peptide)
QFLKEGQLAAGTCEIVTLDRDSSQPRRTIARQTARCACRKGQIAGTTRARPACVDARIIKTKQWCDMLPCLEGEGCDLLINRSGWTCTQPGGRIKTTTVS

SEQ ID NO: 143 - DNA, 363 bp, Artificial Sequence
  P2-C12 anitbody VH
cagtcgctggaggagtccgggggtcgcctggtcacgcctgggacacccctgacactcacctgcaccgtctctggattctccctcagtacctatgcagtgacctgggtccgccaggctccagggaaggggctggaatggatcggatacattaattggcgtggtgggacatcctacgcgaactgggcgaaaggccgattcaccatctccaaaacctcgtcgaccacggtggatctgaaaatgaccagtccgacaaccgaggacacggccacctatttctgtgccagagatgctagtagtggtgctgcttttgggtcttacggcatggacccctggggcccagggaccctcgtcaccgtctcttca

SEQ ID NO: 144 - DNA, 330 bp, Artificial Sequence
  P2-C12 anitbody VH
gagctcgatatgacccagactccatcctccgtgtctgcagctgtgggaggcacagtcaccatcaagtgccaggccagtcagagcattagtagctacttatcctggtatcagcagaaaccagggcagcctcccaagctcctgatctatgaagcatccaaactggcctctggggtcccatcgcggttcagcggcagtggatatgggacagagttcactctcaccatcagcgacctggagtgtgccgatgctgccacttactactgtcaacagggttatagtagtactaatgtttggaatgctttcggcggaggcaccaatgtggaaatcaaa

SEQ ID NO: 145 - protein, 451 aa, Artificial Sequence
  P2-C12 HC
QSLEESGGRLVTPGTPLTLTCTVSGFSLSTYAVTWVRQAPGKGLEWIGYINWRGGTSYANWAKGRFTISKTSSTTVDLKMTSPTTEDTATYFCARDASSGAAFGSYGMDPWGPGTLVTVSSASTKGPSVFPLAPSSKSTSGGTAALGCLVKDYFPEPVTVSWNSGALTSGVHTFPAVLQSSGLYSLSSVVTVPSSSLGTQTYICNVNHKPSNTKVDKKVEPKSCDKTHTCPPCPAPELLGGPSVFLFPPKPKDTLMISRTPEVTCVVVDVSHEDPEVKFNWYVDGVEVHNAKTKPREEQYNSTYRVVSVLTVLHQDWLNGKEYKCKVSNKALPAPIEKTISKAKGQPREPQVYTLPPSREEMTKNQVSLTCLVKGFYPSDIAVEWESNGQPENNYKTTPPVLDSDGSFFLYSKLTVDKSRWQQGNVFSCSVMHEALHNHYTQKSLSLSPGK

SEQ ID NO: 146 - protein, 448 aa, Artificial Sequence
  13B4 HC
QVQLQESGPGLVKPSGTLSLNCAVSGGSISSSNWWSWVRQPPGKGLEWIGEIYHGGTTNYNPSLKGRVTMSVDKTKNQFSLRLSSVTAVDTAVYYCARWQLVGGLDVWGQGTTVTVSSASTKGPSVFPLAPSSKSTSGGTAALGCLVKDYFPEPVTVSWNSGALTSGVHTFPAVLQSSGLYSLSSVVTVPSSSLGTQTYICNVNHKPSNTKVDKKVEPKSCDKTHTCPPCPAPELLGGPSVFLFPPKPKDTLMISRTPEVTCVVVDVSHEDPEVKFNWYVDGVEVHNAKTKPREEQYNSTYRVVSVLTVLHQDWLNGKEYKCKVSNKALPAPIEKTISKAKGQPREPQVYTLPPSREEMTKNQVSLTCLVKGFYPSDIAVEWESNGQPENNYKTTPPVLDSDGSFFLYSKLTVDKSRWQQGNVFSCSVMHEALHNHYTQKSLSLSPGK

SEQ ID NO: 147 - protein, 453 aa, Artificial Sequence
  13F7 HC
QVQLQEWGAGLLKPSETLSLTCAINAESFNGYSWTWIRQTPGKGLEWIGEISHFGSANYNPSLKSRATISADKSKNQFSLKLTSVTAVDTAVYYCARALRGTYSRFYYGMDVWGQGTTVTVSSASTKGPSVFPLAPSSKSTSGGTAALGCLVKDYFPEPVTVSWNSGALTSGVHTFPAVLQSSGLYSLSSVVTVPSSSLGTQTYICNVNHKPSNTKVDKKVEPKSCDKTHTCPPCPAPELLGGPSVFLFPPKPKDTLMISRTPEVTCVVVDVSHEDPEVKFNWYVDGVEVHNAKTKPREEQYNSTYRVVSVLTVLHQDWLNGKEYKCKVSNKALPAPIEKTISKAKGQPREPQVYTLPPSREEMTKNQVSLTCLVKGFYPSDIAVEWESNGQPENNYKTTPPVLDSDGSFFLYSKLTVDKSRWQQGNVFSCSVMHEALHNHYTQKSLSLSPGK

SEQ ID NO: 148 - protein, 450 aa, Artificial Sequence
  15A9 HC
QVQLQESGPGLVKPSETLSLTCTVSGGSISSYYWSWIRQPPGKGLEWIGYIYPSGSTNYNPSLKSRVTISVDTSKNQFSLNLKSVTAVDTAVYYCARVNPFGYYYAMDVWGQGTTVTVSSASTKGPSVFPLAPSSKSTSGGTAALGCLVKDYFPEPVTVSWNSGALTSGVHTFPAVLQSSGLYSLSSVVTVPSSSLGTQTYICNVNHKPSNTKVDKKVEPKSCDKTHTCPPCPAPELLGGPSVFLFPPKPKDTLMISRTPEVTCVVVDVSHEDPEVKFNWYVDGVEVHNAKTKPREEQYNSTYRVVSVLTVLHQDWLNGKEYKCKVSNKALPAPIEKTISKAKGQPREPQVYTLPPSREEMTKNQVSLTCLVKGFYPSDIAVEWESNGQPENNYKTTPPVLDSDGSFFLYSKLTVDKSRWQQGNVFSCSVMHEALHNHYTQKSLSLSPGK

SEQ ID NO: 149 - protein, 446 aa, Artificial Sequence
  P1-A03 HC
QSVEESGGRLVTPGTPLTLTCTVSGFSLSSDYMSWVRQAPGEGLEWIGIIYPSTTTYYASWAKGRFTISKTSSTTVELKMTSLTTEDTATYFCARGSNWSSGMNLWGPGTLVTVSSASTKGPSVFPLAPSSKSTSGGTAALGCLVKDYFPEPVTVSWNSGALTSGVHTFPAVLQSSGLYSLSSVVTVPSSSLGTQTYICNVNHKPSNTKVDKKVEPKSCDKTHTCPPCPAPELLGGPSVFLFPPKPKDTLMISRTPEVTCVVVDVSHEDPEVKFNWYVDGVEVHNAKTKPREEQYNSTYRVVSVLTVLHQDWLNGKEYKCKVSNKALPAPIEKTISKAKGQPREPQVYTLPPSREEMTKNQVSLTCLVKGFYPSDIAVEWESNGQPENNYKTTPPVLDSDGSFFLYSKLTVDKSRWQQGNVFSCSVMHEALHNHYTQKSLSLSPGK

SEQ ID NO: 150 - protein, 443 aa, Artificial Sequence
  P1-A08 HC
QSLEESGGRLVTPGTPLTLTCTASGFSLSTYYMSWVRQAPGKGLEWIGIVYPSGTTYYANWAKGRFTISTASTTVDLMITSPTTEDTATYFCARGDSFGYGLWGPGTLVTVSSASTKGPSVFPLAPSSKSTSGGTAALGCLVKDYFPEPVTVSWNSGALTSGVHTFPAVLQSSGLYSLSSVVTVPSSSLGTQTYICNVNHKPSNTKVDKKVEPKSCDKTHTCPPCPAPELLGGPSVFLFPPKPKDTLMISRTPEVTCVVVDVSHEDPEVKFNWYVDGVEVHNAKTKPREEQYNSTYRVVSVLTVLHQDWLNGKEYKCKVSNKALPAPIEKTISKAKGQPREPQVYTLPPSREEMTKNQVSLTCLVKGFYPSDIAVEWESNGQPENNYKTTPPVLDSDGSFFLYSKLTVDKSRWQQGNVFSCSVMHEALHNHYTQKSLSLSPGK

SEQ ID NO: 151 - protein, 452 aa, Artificial Sequence
  P1-F02 HC
QSLEESGGRLVTPGTPLTLTCTASGFSLSNYYMGWVRQAPGEGLEWIGIIYASGSTYYASWAKGRFTISKTSTTVDLKMTSLTTEDTATYFCARIDIGVGDYGWAYDRLDLWGQGTLVTVSSASTKGPSVFPLAPSSKSTSGGTAALGCLVKDYFPEPVTVSWNSGALTSGVHTFPAVLQSSGLYSLSSVVTVPSSSLGTQTYICNVNHKPSNTKVDKKVEPKSCDKTHTCPPCPAPELLGGPSVFLFPPKPKDTLMISRTPEVTCVVVDVSHEDPEVKFNWYVDGVEVHNAKTKPREEQYNSTYRVVSVLTVLHQDWLNGKEYKCKVSNKALPAPIEKTISKAKGQPREPQVYTLPPSREEMTKNQVSLTCLVKGFYPSDIAVEWESNGQPENNYKTTPPVLDSDGSFFLYSKLTVDKSRWQQGNVFSCSVMHEALHNHYTQKSLSLSPGK

SEQ ID NO: 152 - protein, 451 aa, Artificial Sequence
  P2-A01 HC
QEQLVESGGRLVTPGTPLTLSCTASGFFLSGYYMSWVRQAPGKGLEWIGIIYPSGSTDYASWAKGRFTISKTSTTVDLKITTPTTEDTATYFCARVAGYVGYGYETFFDIWGPGTLVTVSLASTKGPSVFPLAPSSKSTSGGTAALGCLVKDYFPEPVTVSWNSGALTSGVHTFPAVLQSSGLYSLSSVVTVPSSSLGTQTYICNVNHKPSNTKVDKKVEPKSCDKTHTCPPCPAPELLGGPSVFLFPPKPKDTLMISRTPEVTCVVVDVSHEDPEVKFNWYVDGVEVHNAKTKPREEQYNSTYRVVSVLTVLHQDWLNGKEYKCKVSNKALPAPIEKTISKAKGQPREPQVYTLPPSREEMTKNQVSLTCLVKGFYPSDIAVEWESNGQPENNYKTTPPVLDSDGSFFLYSKLTVDKSRWQQGNVFSCSVMHEALHNHYTQKSLSLSPGK

SEQ ID NO: 153 - protein, 446 aa, Artificial Sequence
  P2-A03 HC
QSVEESGGRLVTPGTPLTLTCTVSGFSLNNYDMSWVRQAPGKGLEYIGFMDTDGSAYYATWAKGRFTISRTSTTVDLKMTSPTTEDTATYFCARRGSSYYGGIDIWGPGTPVTVSLASTKGPSVFPLAPSSKSTSGGTAALGCLVKDYFPEPVTVSWNSGALTSGVHTFPAVLQSSGLYSLSSVVTVPSSSLGTQTYICNVNHKPSNTKVDKKVEPKSCDKTHTCPPCPAPELLGGPSVFLFPPKPKDTLMISRTPEVTCVVVDVSHEDPEVKFNWYVDGVEVHNAKTKPREEQYNSTYRVVSVLTVLHQDWLNGKEYKCKVSNKALPAPIEKTISKAKGQPREPQVYTLPPSREEMTKNQVSLTCLVKGFYPSDIAVEWESNGQPENNYKTTPPVLDSDGSFFLYSKLTVDKSRWQQGNVFSCSVMHEALHNHYTQKSLSLSPGK

SEQ ID NO: 154 - protein, 443 aa, Artificial Sequence
  P2-F07 HC
QSLEESGGRLVTPGTPLTLTCTASGFSLSSYYMNWVRQAPGKGLEWIGIIYPSGTTYYAGWAKGRFTISKTSTTVDLKITSPTSEDTATYFCARTVSGYFDIWGPGTLVTVSLASTKGPSVFPLAPSSKSTSGGTAALGCLVKDYFPEPVTVSWNSGALTSGVHTFPAVLQSSGLYSLSSVVTVPSSSLGTQTYICNVNHKPSNTKVDKKVEPKSCDKTHTCPPCPAPELLGGPSVFLFPPKPKDTLMISRTPEVTCVVVDVSHEDPEVKFNWYVDGVEVHNAKTKPREEQYNSTYRVVSVLTVLHQDWLNGKEYKCKVSNKALPAPIEKTISKAKGQPREPQVYTLPPSREEMTKNQVSLTCLVKGFYPSDIAVEWESNGQPENNYKTTPPVLDSDGSFFLYSKLTVDKSRWQQGNVFSCSVMHEALHNHYTQKSLSLSPGK

SEQ ID NO: 155 - protein, 444 aa, Artificial Sequence
  P2-F11 HC
QEQLVESGGRLVTPGTTLTLTCTVSGFSLSSYGVSWVRQAPGKGLEWIGYIANNYNPHYASWAKGRFTISKTSSTTVDLKMTSLTTEDTATYFCARDNYGMDPWGPGTLVTVSSASTKGPSVFPLAPSSKSTSGGTAALGCLVKDYFPEPVTVSWNSGALTSGVHTFPAVLQSSGLYSLSSVVTVPSSSLGTQTYICNVNHKPSNTKVDKKVEPKSCDKTHTCPPCPAPELLGGPSVFLFPPKPKDTLMISRTPEVTCVVVDVSHEDPEVKFNWYVDGVEVHNAKTKPREEQYNSTYRVVSVLTVLHQDWLNGKEYKCKVSNKALPAPIEKTISKAKGQPREPQVYTLPPSREEMTKNQVSLTCLVKGFYPSDIAVEWESNGQPENNYKTTPPVLDSDGSFFLYSKLTVDKSRWQQGNVFSCSVMHEALHNHYTQKSLSLSPGK

SEQ ID NO: 156 - protein, 217 aa, Artificial Sequence
  P2-C12 LC
ELDMTQTPSSVSAAVGGTVTIKCQASQSISSYLSWYQQKPGQPPKLLIYEASKLASGVPSRFSGSGYGTEFTLTISDLECADAATYYCQQGYSSTNVWNAFGGGTNVEIKRSVAAPSVFIFPPSDEQLKSGTASVVCLLNNFYPREAKVQWKVDNALQSGNSQESVTEQDSKDSTYSLSSTLTLSKADYEKHKVYACEVTHQGLSSPVTKSFNRGEC

SEQ ID NO: 157 - protein, 213 aa, Artificial Sequence
  13B4 LC
SYELTQPLSVSVSPGQTASITCSGDKLGNVYASWYQQKPGQSPTLVIYQDNKRPSGIPERFSGSNSGKTATLTISGTQALDEADYYCQAWDSSTAVFGGGTKLTVLRSVAAPSVFIFPPSDEQLKSGTASVVCLLNNFYPREAKVQWKVDNALQSGNSQESVTEQDSKDSTYSLSSTLTLSKADYEKHKVYACEVTHQGLSSPVTKSFNRGEC

SEQ ID NO: 158 - protein, 219 aa, Artificial Sequence
  13F7 LC
DIVMTQTPLSLPVAPGEPASISCRSSQSLLHSNGYNYLDWYVQKPGQPPQLLIYLGSNRASGVPDRFSGSGSGTDFTLKISRVEAEDVGVYYCMQARQTPLTFGGGTKVEIKRSVAAPSVFIFPPSDEQLKSGTASVVCLLNNFYPREAKVQWKVDNALQSGNSQESVTEQDSKDSTYSLSSTLTLSKADYEKHKVYACEVTHQGLSSPVTKSFNRGEC

SEQ ID NO: 159 - protein, 214 aa, Artificial Sequence
  15A9 LC
DIQMTQSPSSLSASVGDRITISCRASQSISTSLNWYQQTPGKAPRLLIYGASTLQSGVPSRFSGGGSGTDFSLTITSLQPEDFATYYCQESASIPRTFGQGTKLDIKRSVAAPSVFIFPPSDEQLKSGTASVVCLLNNFYPREAKVQWKVDNALQSGNSQESVTEQDSKDSTYSLSSTLTLSKADYEKHKVYACEVTHQGLSSPVTKSFNRGEC

SEQ ID NO: 160 - protein, 217 aa, Artificial Sequence
  P1-A03 LC
ELVMTQTPPSLSASVGETVRIRCLASEDIYSGISWYQQKPEKPPTLLISGASNLESGVPPRFSGSGSGTDYTLTIGGVQAEDAATYYCLGGYSYSSTGLTFGAGTNVEIKRSVAAPSVFIFPPSDEQLKSGTASVVCLLNNFYPREAKVQWKVDNALQSGNSQESVTEQDSKDSTYSLSSTLTLSKADYEKHKVYACEVTHQGLSSPVTKSFNRGEC

SEQ ID NO: 161 - protein, 217 aa, Artificial Sequence
  P1-A08 LC
ELVLTQSPSVQVNLGQTVSLTCTADTLSRSYASWYQQKPGQAPVLLIYRDTSRPSGVPDRFSGSSSGNTATLTISGAQAGDEADYYCATSDGSGSNYQYVFGGGTQLTVTRSVAAPSVFIFPPSDEQLKSGTASVVCLLNNFYPREAKVQWKVDNALQSGNSQESVTEQDSKDSTYSLSSTLTLSKADYEKHKVYACEVTHQGLSSPVTKSFNRGEC

SEQ ID NO: 162 - protein, 215 aa, Artificial Sequence
  P1-F02 LC
ELDMTQTPPSLSASVGETVRIRCLASEDIYSGISWYQQKPGKPPTLLIYGASNLESGVPPRFSGSGSGTDYTLTIGGVQAEDAATYYCLGGYSYSSITFGAGTNVEIKRSVAAPSVFIFPPSDEQLKSGTASVVCLLNNFYPREAKVQWKVDNALQSGNSQESVTEQDSKDSTYSLSSTLTLSKADYEKHKVYACEVTHQGLSSPVTKSFNRGEC

SEQ ID NO: 163 - protein, 219 aa, Artificial Sequence
  P2-A01 LC
ELVMTQTPPSLSASVGETVRIRCLASEDIYSGISWYQQKPGKPPTLLIYGASNLESGVPPRFSGSGSGSDYTLTIGGVQAEDAATYYCLGGVTYSSTGTHLTFGAGTNVEIKRSVAAPSVFIFPPSDEQLKSGTASVVCLLNNFYPREAKVQWKVDNALQSGNSQESVTEQDSKDSTYSLSSTLTLSKADYEKHKVYACEVTHQGLSSPVTKSFNRGEC

SEQ ID NO: 164 - protein, 219 aa, Artificial Sequence
  P2-A03 LC
ELDLTQTPASVSEPVGGTVTIKCQASQSIGGNLAWYQQKPGQPPKLLIYRASTLASGVPSRFKGSGSGTDFTLTISDLECADAATYYCQSPAYDPAAYVGNAFGGGTELEILRSVAAPSVFIFPPSDEQLKSGTASVVCLLNNFYPREAKVQWKVDNALQSGNSQESVTEQDSKDSTYSLSSTLTLSKADYEKHKVYACEVTHQGLSSPVTKSFNRGEC

SEQ ID NO: 165 - protein, 214 aa, Artificial Sequence
  P2-F07 LC
ELDLTQTPPSLSASVGGTVTINCLASEDIYSALAWYQQKPGKPPTLLISGTSNLESGVPPRFSGSGSGTDYTLTIGGVQAEDAATYFCQGYSSYPLTFGAGTNVEIKRSVAAPSVFIFPPSDEQLKSGTASVVCLLNNFYPREAKVQWKVDNALQSGNSQESVTEQDSKDSTYSLSSTLTLSKADYEKHKVYACEVTHQGLSSPVTKSFNRGEC

SEQ ID NO: 166 - protein, 220 aa, Artificial Sequence
  P2-F11 LC
ELDLTQTPSSVSAAVGGTVTINCQASQSVYNNKNLAWYQQKPGQPPKLLIYAASTLASGVSSRFKGSGSGTQFTLTISDVQCDDAATYYCQGEFSCSSADCNAFGGGTELEILRSVAAPSVFIFPPSDEQLKSGTASVVCLLNNFYPREAKVQWKVDNALQSGNSQESVTEQDSKDSTYSLSSTLTLSKADYEKHKVYACEVTHQGLSSPVTKSFNRGEC